European Patent Specification EP 3 388 509 B1, published June 17, 2026. Title: ISOLATED RENAL CELLS AND USES THEREOF. Applicant: TENGION, INC. Application DIVISIONAL APPLICATION OF EP 13170810.9. The sequence listing filed with the application follows.

SEQUENCE LISTING (3 sequences)

SEQ ID NO: 1 - DNA, 17 bp, Artificial Sequence
  Description of Artificial Sequence: Synthetic oligonucleotide primer
aagcgccccatgaatgc

SEQ ID NO: 2 - DNA, 19 bp, Artificial Sequence
  Description of Artificial Sequence: Synthetic oligonucleotide primer
agccaacttgcgcctctct

SEQ ID NO: 3 - DNA, 19 bp, Artificial Sequence
  Description of Artificial Sequence: Synthetic oligonucleotide probe
tttatggtgtggtcccgtg